European Patent Specification EP 4 547 840 B1, published November 26, 2025. Title: PROTECTED DNA AND METHODS FOR THE PRODUCTION THEREOF. Applicant: 4basebio UK Ltd. Application WO. The sequence listing filed with the application follows.

SEQUENCE LISTING (28 sequences)

SEQ ID NO: 1 - DNA, 17 bp, synthetic construct
  source 1..17: mol_type = other DNA
  modified_base 1: mod_base = OTHER; note = nuclease resistant nucleotide
nacaaatgttagccctn

SEQ ID NO: 2 - DNA, 17 bp, synthetic construct
  source 1..17: mol_type = other DNA
nagggctaacatttgtn

SEQ ID NO: 3 - DNA, 17 bp, synthetic construct
  source 1..17: mol_type = other DNA
  modified_base 17: mod_base = OTHER; note = nuclease resistant nucleotide
nagggctaacatttgtn

SEQ ID NO: 4 - DNA, 16 bp, synthetic construct
  source 1..16: mol_type = other DNA
  modified_base 16: mod_base = OTHER; note = nuclease resistant nucleotide
ncatgctaacatttgn

SEQ ID NO: 5 - DNA, 16 bp, synthetic construct
  source 1..16: mol_type = other DNA
ncaaatgttagcatgn

SEQ ID NO: 6 - DNA, 16 bp, synthetic construct
  source 1..16: mol_type = other DNA
  modified_base 1: mod_base = OTHER; note = nuclease resistant nucleotide
ncaaatgttagcatgn

SEQ ID NO: 7 - DNA, 12 bp, synthetic construct
  source 1..12: mol_type = other DNA
  modified_base 1: mod_base = OTHER; note = nuclease resistant nucleotide
nacaaatgttag

SEQ ID NO: 8 - DNA, 16 bp, synthetic construct
  source 1..16: mol_type = other DNA
agggctaacatttgtn

SEQ ID NO: 9 - DNA, 16 bp, synthetic construct
  source 1..16: mol_type = other DNA
  modified_base 16: mod_base = OTHER; note = nuclease resistant nucleotide
agggctaacatttgtn

SEQ ID NO: 10 - DNA, 15 bp, synthetic construct
  source 1..15: mol_type = other DNA
  modified_base 15: mod_base = OTHER; note = nuclease resistant nucleotide
catgctaacatttgn

SEQ ID NO: 11 - DNA, 11 bp, synthetic construct
  source 1..11: mol_type = other DNA
ncaaatgttag

SEQ ID NO: 12 - DNA, 11 bp, synthetic construct
  source 1..11: mol_type = other DNA
  modified_base 1: mod_base = OTHER; note = nuclease resistant nucleotide
ncaaatgttag

SEQ ID NO: 13 - DNA, 16 bp, synthetic construct
  source 1..16: mol_type = other DNA
  modified_base 1..5: mod_base = OTHER; note = nuclease resistant nucleotide
ggccaacaaatgttag

SEQ ID NO: 14 - DNA, 20 bp, synthetic construct
  source 1..20: mol_type = other DNA
  modified_base 16..20: mod_base = OTHER; note = nuclease resistant nucleotide
agggctaacatttgttggcc

SEQ ID NO: 15 - DNA, 18 bp, synthetic construct
  source 1..18: mol_type = other DNA
  modified_base 14..18: mod_base = OTHER; note = nuclease resistant nucleotide
aaaaaaaaaaaaaaaaaa

SEQ ID NO: 16 - DNA, 14 bp, synthetic construct
  source 1..14: mol_type = other DNA
  modified_base 1..5: mod_base = OTHER; note = nuclease resistant nucleotide
tttttttttttttt

SEQ ID NO: 17 - DNA, 16 bp, synthetic construct
  source 1..16: mol_type = other DNA
ggccaacaaatgttag

SEQ ID NO: 18 - DNA, 20 bp, synthetic construct
  source 1..20: mol_type = other DNA
agggctaacatttgttggcc

SEQ ID NO: 19 - DNA, 20 bp, synthetic construct
  source 1..20: mol_type = other DNA
  modified_base 6: mod_base = OTHER; note = abasic site
agggcnaacatttgttggcc

SEQ ID NO: 20 - DNA, 20 bp, synthetic construct
  source 1..20: mol_type = other DNA
  modified_base 8: mod_base = OTHER; note = abasic site
agggctancatttgttggcc

SEQ ID NO: 21 - DNA, 20 bp, synthetic construct
  source 1..20: mol_type = other DNA
  modified_base 10: mod_base = OTHER; note = abasic site
agggctaacntttgttggcc

SEQ ID NO: 22 - DNA, 20 bp, synthetic construct
  source 1..20: mol_type = other DNA
  modified_base 14: mod_base = OTHER; note = abasic site
agggctaacatttnttggcc

SEQ ID NO: 23 - DNA, 20 bp, synthetic construct
  source 1..20: mol_type = other DNA
  modified_base 6: mod_base = OTHER; note = uracil
agggctaacatttgttggcc

SEQ ID NO: 24 - DNA, 20 bp, synthetic construct
  source 1..20: mol_type = other DNA
  modified_base 11: mod_base = OTHER; note = uracil
agggctaacatttgttggcc

SEQ ID NO: 25 - DNA, 20 bp, synthetic construct
  source 1..20: mol_type = other DNA
  modified_base 13: mod_base = OTHER; note = uracil
agggctaacatttgttggcc

SEQ ID NO: 26 - DNA, 20 bp, synthetic construct
  source 1..20: mol_type = other DNA
  modified_base 6: mod_base = OTHER; note = uracil
  modified_base 11: mod_base = OTHER; note = uracil
  modified_base 13: mod_base = OTHER; note = uracil
agggctaacatttgttggcc

SEQ ID NO: 27 - DNA, 18 bp, synthetic construct
  source 1..18: mol_type = other DNA
aaaaaaaaaaaaaaaaaa

SEQ ID NO: 28 - DNA, 14 bp, synthetic construct
  source 1..14: mol_type = other DNA
tttttttttttttt